European Patent Application EP 4 406 552 A1, published July 31, 2024. Title: 抗CD40抗体的应用. Applicant: 正大天晴药业集团股份有限公司. The sequence listing filed with the application follows.

SEQUENCE LISTING (43 sequences)

SEQ ID NO: 1 - protein, 5 aa, synthetic construct
  REGION 1..5: note = VH-CDR1 for mouse, chimeric and humanized C1H1 antibodies; note (original language) = 小鼠、嵌合和人源化C1H1抗体的VH-CDR1
NYGIS

SEQ ID NO: 2 - protein, 5 aa, synthetic construct
  REGION 1..5: note = VH-CDR1 for mouse and chimeric 1A3 antibodies; note (original language) = 小鼠和嵌合1A3抗体的VH-CDR1
GYYLH

SEQ ID NO: 3 - protein, 5 aa, synthetic construct
  REGION 1..5: note = VH-CDR1 for mouse and chimeric 1D1 antibodies; note (original language) = 小鼠和嵌合1D1抗体的VH-CDR1
DYVMH

SEQ ID NO: 4 - protein, 17 aa, synthetic construct
  REGION 1..17: note = VH-CDR2 for mouse, chimeric and humanized C1H1 antibodies; note (original language) = 小鼠、嵌合和人源化C1H1抗体的VH-CDR2
SISSGGDNTYYPDNVKG

SEQ ID NO: 5 - protein, 17 aa, synthetic construct
  REGION 1..17: note = VH-CDR2 for mouse and chimeric 1A3 antibodies; note (original language) = 小鼠和嵌合1A3抗体的VH-CDR2
YISCHDGTIIYNQKFKG

SEQ ID NO: 6 - protein, 17 aa, synthetic construct
  REGION 1..17: note = VH-CDR2 for mouse and chimeric 1D1 antibodies; note (original language) = 小鼠和嵌合1D1抗体的VH-CDR2
YINPYNDGTTYNEKFKG

SEQ ID NO: 7 - protein, 8 aa, synthetic construct
  REGION 1..8: note = VH-CDR3 for mouse, chimeric and humanized C1H1 antibodies; note (original language) = 小鼠、嵌合和人源化C1H1抗体的VH-CDR3
AGEKAMDY

SEQ ID NO: 8 - protein, 13 aa, synthetic construct
  REGION 1..13: note = VH-CDR3 for mouse and chimeric 1A3 antibodies; note (original language) = 小鼠和嵌合1A3抗体的VH-CDR3
FLNYYGSNYAMDY

SEQ ID NO: 9 - protein, 10 aa, synthetic construct
  REGION 1..10: note = VH-CDR3 for mouse and chimeric 1D1 antibodies; note (original language) = 小鼠和嵌合1D1抗体的VH-CDR3
GFLRESWFGY

SEQ ID NO: 10 - protein, 11 aa, synthetic construct
  REGION 1..11: note = VL-CDR1 for mouse, chimeric and humanized C1H1 antibodies; note (original language) = 小鼠、嵌合和人源化C1H1抗体的VL-CDR1
RASQTINNNLH

SEQ ID NO: 11 - protein, 11 aa, synthetic construct
  REGION 1..11: note = VL-CDR1 for mouse and chimeric 1A3 antibodies; note (original language) = 小鼠和嵌合1A3抗体的VL-CDR1
KASQDVGPAVA

SEQ ID NO: 12 - protein, 16 aa, synthetic construct
  REGION 1..16: note = VL-CDR1 for mouse and chimeric 1D1 antibodies; note (original language) = 小鼠和嵌合1D1抗体的VL-CDR1
RSSQNIVHSNGNTYLD

SEQ ID NO: 13 - protein, 7 aa, synthetic construct
  REGION 1..7: note = VL-CDR2 for mouse, chimeric and humanized C1H1 antibody; note (original language) = 小鼠、嵌合和人源化C1H1抗体的VL-CDR2
YASQSIS

SEQ ID NO: 14 - protein, 7 aa, synthetic construct
  REGION 1..7: note = VL-CDR2 for mouse and chimeric 1A3 antibodies; note (original language) = 小鼠和嵌合1A3抗体的VL-CDR2
WASTRHT

SEQ ID NO: 15 - protein, 7 aa, synthetic construct
  REGION 1..7: note = VL-CDR2 for mouse and chimeric 1D1 antibodies; note (original language) = 小鼠和嵌合1D1抗体的VL-CDR2
KVSNRFS

SEQ ID NO: 16 - protein, 9 aa, synthetic construct
  REGION 1..9: note = VL-CDR3 for mouse, chimeric and humanized C1H1 antibodies; note (original language) = 小鼠、嵌合和人源化C1H1抗体的VL-CDR3
QQFSSWPLT

SEQ ID NO: 17 - protein, 9 aa, synthetic construct
  REGION 1..9: note = VL-CDR3 for mouse and chimeric 1A3 antibodies; note (original language) = 小鼠和嵌合1A3抗体的VL-CDR3
QQYFTYPLT

SEQ ID NO: 18 - protein, 9 aa, synthetic construct
  REGION 1..9: note = VL-CDR3 for mouse and chimeric 1D1 antibodies; note (original language) = 小鼠和嵌合1D1抗体的VL-CDR3
FQGSHVPPT

SEQ ID NO: 19 - protein, 117 aa, synthetic construct
  REGION 1..117: note = VH for mouse and chimeric C1H1 antibodies; note (original language) = 小鼠和嵌合C1H1抗体的VH
EVKLVESGGGLVKPGASLKLSCAASGFTFSNYGISWVRQTSDKRLEWVASISSGGDNTYYPDNVKGRFTISRENAKNTLYLQMSSLKSEDTALYYCARAGEKAMDYWGQGTSVTVSS

SEQ ID NO: 20 - protein, 117 aa, synthetic construct
  REGION 1..117: note = VH for huC1H1-V1 to huC1H1-V4; note (original language) = huC1H1-V1 至 huC1H1-V4的VH
  VARIANT 49: note = X can be A or S; note (original language) = X 可以是 A 或 S
EVQLVESGGGLVKPGGSLRLSCAASGFTFSNYGISWVRQAPGKGLEWVXSISSGGDNTYYPDNVKGRFTISRDNAKNSLYLQMNSLRAEDTAVYYCARAGEKAMDYWGQGTLVTVSS

SEQ ID NO: 21 - protein, 122 aa, synthetic construct
  REGION 1..122: note = VH for mouse and chimeric 1A3 antibodies; note (original language) = 小鼠和嵌合1A3抗体的VH
EVQLQQSGPELVKTGASVKISCKASGYSFIGYYLHWVKQSLGKGLEWIGYISCHDGTIIYNQKFKGKATFTLDTSSSTAYMQFSSLTSEDSAVYFCARFLNYYGSNYAMDYWGQGTSVTVSS

SEQ ID NO: 22 - protein, 119 aa, synthetic construct
  REGION 1..119: note = VH for mouse and chimeric 1D1 antibodies; note (original language) = 小鼠和嵌合1D1抗体的VH
EVQLQQSGPELVKPGASVKMSCKASGYTFTDYVMHWVKQKPGQGLECIGYINPYNDGTTYNEKFKGKATLTSDKSSNAAYLELSSLTSEDSAVYYCARGFLRESWFGYWGQGTLVTVSA

SEQ ID NO: 23 - protein, 107 aa, synthetic construct
  REGION 1..107: note = VL for mouse and chimeric C1H1 antibodies; note (original language) = 小鼠和嵌合C1H1抗体的VL
DIVLTQSPVTLSVTPGDSVSLSCRASQTINNNLHWYQQKSHESPRLLIKYASQSISGIPSRFSGSGSGTDFTLSINSVETEDFGIYFCQQFSSWPLTFGAGTKLELK

SEQ ID NO: 24 - protein, 107 aa, synthetic construct
  REGION 1..107: note = VL for huC1H1-V1 to huC1H1-V4; note (original language) = huC1H1-V1 至 huC1H1-V4的VL
  VARIANT 49: note = X can be K or Y; note (original language) = X 可以是 K 或 Y
  VARIANT 87: note = X can be F or Y; note (original language) = X 可以是 F 或 Y
EIVLTQSPATLSLSPGERATLSCRASQTINNNLHWYQQKPGQAPRLLIXYASQSISGIPARFSGSGSGTDFTLTISSLEPEDFAVYXCQQFSSWPLTFGGGTKVEIK

SEQ ID NO: 25 - protein, 107 aa, synthetic construct
  REGION 1..107: note = VL for mouse and chimeric 1A3 antibodies; note (original language) = 小鼠和嵌合1A3抗体的VL
DIVMTQSHKFMSTSVGDRVSITCKASQDVGPAVAWYQQKPGQSPKLLIYWASTRHTGVPDRFTGSGYGTDFTLTINNVQSEDLADYFCQQYFTYPLTFGGGTKLEIK

SEQ ID NO: 26 - protein, 112 aa, synthetic construct
  REGION 1..112: note = VL for mouse and chimeric 1D1 antibodies; note (original language) = 小鼠和嵌合1D1抗体的VL
DVLLTQTPLSLPVSLGDQASISCRSSQNIVHSNGNTYLDWYLQKPGQSPKLLIYKVSNRFSGVPDRFSGSGSGTDFTLKISRVEAEDLGVYYCFQGSHVPPTFGGGTKLELK

SEQ ID NO: 27 - protein, 330 aa, synthetic construct
  REGION 1..330: note = Heavy chain constant region for chimeric antibodies; note (original language) = 嵌合抗体的重链恒定区
ASTKGPSVFPLAPSSKSTSGGTAALGCLVKDYFPEPVTVSWNSGALTSGVHTFPAVLQSSGLYSLSSVVTVPSSSLGTQTYICNVNHKPSNTKVDKKVEPKSCDKTHTCPPCPAPELLGGPSVFLFPPKPKDTLMISRTPEVTCVVVDVSHEDPEVKFNWYVDGVEVHNAKTKPREEQYNSTYRVVSVLTVLHQDWLNGKEYKCKVSNKALPAPIEKTISKAKGQPREPQVYTLPPSREEMTKNQVSLTCLVKGFYPSDIAVEWESNGQPENNYKTTPPVLDSDGSFFLYSKLTVDKSRWQQGNVFSCSVMHEALHNHYTQKSLSLSPGK

SEQ ID NO: 28 - protein, 326 aa, synthetic construct
  REGION 1..326: note = Heavy chain constant region for humanized antibodies; note (original language) = 人源化抗体的重链恒定区
ASTKGPSVFPLAPCSRSTSESTAALGCLVKDYFPEPVTVSWNSGALTSGVHTFPAVLQSSGLYSLSSVVTVPSSNFGTQTYTCNVDHKPSNTKVDKTVERKCCVECPPCPAPPVAGPSVFLFPPKPKDTLMISRTPEVTCVVVDVSHEDPEVQFNWYVDGVEVHNAKTKPREEQFNSTFRVVSVLTVVHQDWLNGKEYKCKVSNKGLPAPIEKTISKTKGQPREPQVYTLPPSREEMTKNQVSLTCLVKGFYPSDIAVEWESNGQPENNYKTTPPMLDSDGSFFLYSKLTVDKSRWQQGNVFSCSVMHEALHNHYTQKSLSLSPGK

SEQ ID NO: 29 - protein, 107 aa, synthetic construct [sequence omitted]

SEQ ID NO: 30 - protein, 277 aa, Homo sapiens
MVRLPLQCVLWGCLLTAVHPEPPTACREKQYLINSQCCSLCQPGQKLVSDCTEFTETECLPCGESEFLDTWNRETHCHQHKYCDPNLGLRVQQKGTSETDTICTCEEGWHCTSEACESCVLHRSCSPGFGVKQIATGVSDTICEPCPVGFFSNVSSAFEKCHPWTSCETKDLVVQQAGTNKTDVVCGPQDRLRALVVIPIIFGILFAILLVLVFIKKVAKKPTNKAPHPKQEPQEINFPDDLPGSNTAAPVQETLHGCQPVTQEDGKESRISVQERQ

SEQ ID NO: 31 - DNA, 351 bp, synthetic construct
  gene 1..351: note = VH for mouse C1H1; note (original language) = 小鼠C1H1抗体的VH
  source 1..351: mol_type = other DNA
gaagtgaaactggtggagtctgggggaggcttagtgaagcctggagcgtctctgaaactctcctgtgcagcctctggattcactttcagtaactatggcatatcttgggttcgccagacttcagacaagaggctggagtgggtcgcatccattagtagtggtggtgataacacctactatccagacaatgtaaagggccgattcaccatctccagagagaatgccaagaacaccctatacctacaaatgagtagtctgaagtctgaggacacggccttgtattactgtgcaagagctggggagaaggctatggactactggggtcaaggaacctcagtcaccgtctcctca

SEQ ID NO: 32 - DNA, 351 bp, synthetic construct
  gene 1..351: note = VH for chimeric C1H1; note (original language) = 嵌合C1H1抗体的VH
  source 1..351: mol_type = other DNA
gaggtgaagctggtggagtccggcggcggcctggtgaagcctggagctagcctgaagctgagctgcgccgccagcggcttcaccttttccaactacggcatcagctgggtgaggcagacaagcgataagaggctggagtgggtggccagcatcagcagcggcggcgataacacatactaccctgacaacgtgaagggcagattcaccatcagcagggagaacgccaagaataccctgtacctgcagatgagcagcctgaagagcgaggacaccgccctgtactactgtgccagggccggcgagaaggccatggactactggggccagggcacctccgtgaccgtgagctcc

SEQ ID NO: 33 - DNA, 351 bp, synthetic construct
  gene 1..351: note = VH for huC1H1-V2 and huC1H1-V4; note (original language) = huC1H1-V2 和 huC1H1-V4的VH
  source 1..351: mol_type = other DNA
gaggtgcagctggtggagagcggcggcggactggtgaagcctggcggaagcctgagactgagctgcgccgcctccggcttcaccttctccaactacggcatcagctgggtgaggcaggcccccggaaagggcctggagtgggtgagcagcatcagcagcggcggcgacaatacctactaccctgacaacgtgaagggcaggttcaccatcagcagagacaatgccaagaattccctgtacctgcagatgaacagcctgagagccgaggatacagccgtgtactactgtgccagagccggcgagaaggccatggattactggggccagggcaccctggtgaccgtgtcctcc

SEQ ID NO: 34 - DNA, 321 bp, synthetic construct
  gene 1..321: note = VL for mouse C1H1; note (original language) = 小鼠C1H1抗体的VL
  source 1..321: mol_type = other DNA
gatattgtactaactcagtctccagtcaccctgtctgtgactccaggagatagcgtcagtctttcctgcagggccagccaaactattaacaacaacctacactggtatcaacaaaaatcacatgagtctccaaggcttctcatcaagtatgcttcccagtccatctctgggatcccctccaggttcagtggcagtggatcagggacagatttcactctcagtatcaacagtgtggagactgaagattttggaatatatttctgtcaacagtttagcagctggcctcttacgttcggtgctgggactaagctggagctgaaa

SEQ ID NO: 35 - DNA, 321 bp, synthetic construct
  gene 1..321: note = VL for chimeric C1H1; note (original language) = 嵌合C1H1抗体的VL
  source 1..321: mol_type = other DNA
gatatcgtgctgacccagagccccgtgaccctgagcgtgacacccggcgacagcgtgagcctgtcctgcagagccagccagaccatcaacaacaatctgcactggtatcaacagaagagccacgagagccccaggctgctgatcaagtacgccagccagagcatctccggcatccctagcagattcagcggctccggctccggcacagactttaccctgagcatcaacagcgtggagaccgaggatttcggcatctacttttgccagcagttttcctcctggcctctgacattcggcgccggcacaaagctggagctgaag

SEQ ID NO: 36 - DNA, 321 bp, synthetic construct
  gene 1..321: note = VL for huC1H1-V1 and huC1H1-V2; note (original language) = huC1H1-V1 和 huC1H1-V2的VL
  source 1..321: mol_type = other DNA
gagatcgtgctgacccagagccccgccaccctgagcctgagccctggagagagggccaccctgtcctgcagggcctcccagacaatcaataataatctgcactggtatcaacagaagcccggccaggcccccaggctgctgatcaagtacgccagccagtccatcagcggcatccctgccaggttctccggcagcggcagcggaacagacttcaccctgaccatctcctccctggagcctgaggactttgccgtgtacttttgccagcagttctccagctggcctctgacctttggcggcggcaccaaggtggagatcaag

SEQ ID NO: 37 - DNA, 993 bp, synthetic construct
  gene 1..993: note = Heavy chain constant region for chimeric antibodies; note (original language) = 嵌合抗体的重链恒定区
  source 1..993: mol_type = other DNA
gctagcaccaagggcccatcggtcttccccctggcaccctcctccaagagcacctctgggggcacagcggccctgggctgcctggtcaaggactacttccccgaaccggtgacggtgtcgtggaactcaggcgccctgaccagcggcgtgcacaccttcccggctgtcctacagtcctcaggactctactccctcagcagcgtggtgaccgtgccctccagcagcttgggcacccagacctacatctgcaacgtgaatcacaagcccagcaacaccaaggtggacaagaaagttgagcccaaatcttgtgacaaaactcacacatgcccaccgtgcccagcacctgaactcctggggggaccgtcagtcttcctcttccccccaaaacccaaggacaccctcatgatctcccggacccctgaggtcacatgcgtggtggtggacgtgagccacgaagaccctgaggtcaagttcaactggtacgtggacggcgtggaggtgcataatgccaagacaaagccgcgggaggagcagtacaacagcacgtaccgtgtggtcagcgtcctcaccgtcctgcaccaggactggctgaatggcaaggagtacaagtgcaaggtctccaacaaagccctcccagcccccatcgagaaaaccatctccaaagccaaagggcagccccgagaaccacaggtgtacaccctgcccccatcccgggaggagatgaccaagaaccaggtcagcctgacctgcctggtcaaaggcttctatcccagcgacatcgccgtggagtgggagagcaatgggcagccggagaacaactacaagaccacgcctcccgtgctggactccgacggctccttcttcctctacagcaagctcaccgtggacaagagcaggtggcagcaggggaacgtcttctcatgctccgtgatgcatgaggctctgcacaaccactacacgcagaagagcctctccctgtctccgggtaaatga

SEQ ID NO: 38 - DNA, 981 bp, synthetic construct
  gene 1..981: note = Heavy chain constant region for humanized antibodies; note (original language) = 人源化抗体的重链恒定区
  source 1..981: mol_type = other DNA
gcctccaccaagggcccatcggtcttccccctggcgccctgctccaggagcacctctgagagcacagcggccctgggctgcctggtcaaggactacttccccgaaccggtgacggtgtcgtggaactcaggcgctctgaccagcggcgtgcacaccttcccagctgtcctacagtcctcaggactctactccctcagcagcgtggtgaccgtgccctccagcaacttcggcacccagacctacacctgcaacgtagatcacaagcccagcaacaccaaggtggacaagacagttgagcgcaaatgttgtgtcgagtgcccaccgtgcccagcaccacctgtggcaggaccgtcagtcttcctcttccccccaaaacccaaggacaccctcatgatctcccggacccctgaggtcacgtgcgtggtggtggacgtgagccacgaagaccccgaggtccagttcaactggtacgtggacggcgtggaggtgcataatgccaagacaaagccacgggaggagcagttcaacagcacgttccgtgtggtcagcgtcctcaccgttgtgcaccaggactggctgaacggcaaggagtacaagtgcaaggtctccaacaaaggcctcccagcccccatcgagaaaaccatctccaaaaccaaagggcagccccgagaaccacaggtgtacaccctgcccccatcccgggaggagatgaccaagaaccaggtcagcctgacctgcctggtcaaaggcttctaccccagcgacatcgccgtggagtgggagagcaatgggcagccggagaacaactacaagaccacacctcccatgctggactccgacggctccttcttcctctacagcaagctcaccgtggacaagagcaggtggcagcaggggaacgtcttctcatgctccgtgatgcatgaggctctgcacaaccactacacgcagaagagcctctccctgtctccgggtaaatga

SEQ ID NO: 39 - DNA, 324 bp, synthetic construct
  gene 1..324: note = Light chain constant region for chimeric and humanized antibodies; note (original language) = 嵌合和人源化抗体的轻链恒定区
  source 1..324: mol_type = other DNA
cgtacggtggcggcgccatctgtcttcatcttcccgccatctgatgagcagttgaaatctggaactgcctctgttgtgtgcctgctgaataacttctatcccagagaggccaaagtacagtggaaggtggataacgccctccaatcgggtaactcccaggagagtgtcacagagcaggacagcaaggacagcacctacagcctcagcagcaccctgacgctgagcaaagcagactacgagaaacacaaagtctacgcctgcgaagtcacccatcagggcctgagctcgcccgtcacaaagagcttcaacaggggagagtgttga

SEQ ID NO: 40 - protein, 444 aa, synthetic construct
  REGION 1..444: note = Heavy chain of Dacetuzumab; note (original language) = Dacetuzumab的重链
EVQLVESGGGLVQPGGSLRLSCAASGYSFTGYYIHWVRQAPGKGLEWVARVIPNAGGTSYNQKFKGRFTLSVDNSKNTAYLQMNSLRAEDTAVYYCAREGIYWWGQGTLVTVSSASTKGPSVFPLAPSSKSTSGGTAALGCLVKDYFPEPVTVSWNSGALTSGVHTFPAVLQSSGLYSLSSVVTVPSSSLGTQTYICNVNHKPSNTKVDKKVEPKSCDKTHTCPPCPAPELLGGPSVFLFPPKPKDTLMISRTPEVTCVVVDVSHEDPEVKFNWYVDGVEVHNAKTKPREEQYNSTYRVVSVLTVLHQDWLNGKEYKCKVSNKALPAPIEKTISKAKGQPREPQVYTLPPSREEMTKNQVSLTCLVKGFYPSDIAVEWESNGQPENNYKTTPPVLDSDGSFFLYSKLTVDKSRWQQGNVFSCSVMHEALHNHYTQKSLSLSPGK

SEQ ID NO: 41 - protein, 219 aa, synthetic construct
  REGION 1..219: note = Light chain of Dacetuzumab; note (original language) = Dacetuzumab的轻链
DIQMTQSPSSLSASVGDRVTITCRSSQSLVHSNGNTFLHWYQQKPGKAPKLLIYTVSNRFSGVPSRFSGSGSGTDFTLTISSLQPEDFATYFCSQTTHVPWTFGQGTKVEIKRTVAAPSVFIFPPSDEQLKSGTASVVCLLNNFYPREAKVQWKVDNALQSGNSQESVTEQDSKDSTYSLSSTLTLSKADYEKHKVYACEVTHQGLSSPVTKSFNRGEC

SEQ ID NO: 42 - protein, 452 aa, synthetic construct
  REGION 1..452: note = Heavy chain of Selicrelumab; note (original language) = Selicrelumab的重链
QVQLVQSGAEVKKPGASVKVSCKASGYTFTGYYMHWVRQAPGQGLEWMGWINPDSGGTNYAQKFQGRVTMTRDTSISTAYMELNRLRSDDTAVYYCARDQPLGYCTNGVCSYFDYWGQGTLVTVSSASTKGPSVFPLAPCSRSTSESTAALGCLVKDYFPEPVTVSWNSGALTSGVHTFPAVLQSSGLYSLSSVVTVPSSNFGTQTYTCNVDHKPSNTKVDKTVERKCCVECPPCPAPPVAGPSVFLFPPKPKDTLMISRTPEVTCVVVDVSHEDPEVQFNWYVDGVEVHNAKTKPREEQFNSTFRVVSVLTVVHQDWLNGKEYKCKVSNKGLPAPIEKTISKTKGQPREPQVYTLPPSREEMTKNQVSLTCLVKGFYPSDIAVEWESNGQPENNYKTTPPMLDSDGSFFLYSKLTVDKSRWQQGNVFSCSVMHEALHNHYTQKSLSLSPGK

SEQ ID NO: 43 - protein, 214 aa, synthetic construct
  REGION 1..214: note = Light chain of Selicrelumab; note (original language) = Selicrelumab的轻链
DIQMTQSPSSVSASVGDRVTITCRASQGIYSWLAWYQQKPGKAPNLLIYTASTLQSGVPSRFSGSGSGTDFTLTISSLQPEDFATYYCQQANIFPLTFGGGTKVEIKRTVAAPSVFIFPPSDEQLKSGTASVVCLLNNFYPREAKVQWKVDNALQSGNSQESVTEQDSKDSTYSLSSTLTLSKADYEKHKVYACEVTHQGLSSPVTKSFNRGEC